European Patent Specification EP 3 848 025 B9, published August 16, 2023. Title: Compositions comprising amino acids for use in the prevention and treatment of chemotherapy side effects. Applicant: Professional Dietetics International Srl, Professional Dietetics Spa. The sequence listing filed with the application follows.

SEQUENCE LISTING (30 sequences)

SEQ ID NO: 1 - DNA, 23 bp, Artificial Sequence
  Cat Primer Sense 5'-3'
cactgacgagatggcacactttg

SEQ ID NO: 2 - DNA, 22 bp, Artificial Sequence
  Cat Primer Antisense 5'-3'
tggagaaccgaacggcaatagg

SEQ ID NO: 3 - DNA, 24 bp, Artificial Sequence
  COX IV Primer Sense 5'-3'
tgggactatgacaagaatgagtgg

SEQ ID NO: 4 - DNA, 23 bp, Artificial Sequence
  COX IV Primer Antisense 5'-3'
ttagcatggaccattggatacgg

SEQ ID NO: 5 - DNA, 22 bp, Artificial Sequence
  Cyt c Primer Sense 5'-3'
ataggggcatgtcacctcaaac

SEQ ID NO: 6 - DNA, 22 bp, Artificial Sequence
  Primer Antisense 5'-3'
gtggttagccatgacctgaaag

SEQ ID NO: 7 - DNA, 20 bp, Artificial Sequence
  eNOS Primer Sense 5'-3'
agcggctggtacatgagttc

SEQ ID NO: 8 - DNA, 21 bp, Artificial Sequence
  eNOS Primer Antisense 5'-3'
gatgaggttgtcctggtgtcc

SEQ ID NO: 9 - DNA, 19 bp, Artificial Sequence
  GPX1 Primer Sense 5'-3'
tctgggacctcgtggactg

SEQ ID NO: 10 - DNA, 23 bp, Artificial Sequence
  GPX1 Primer Antisense 5'-3'
cacttcgcacttctcaaacaatg

SEQ ID NO: 11 - DNA, 20 bp, Artificial Sequence
  KLF15 Primer Sense 5'-3'
acaccaagagcagccacctc

SEQ ID NO: 12 - DNA, 20 bp, Artificial Sequence
  KLF15 Primer Antisense 5'-3'
tgagatcgccggtgccttga

SEQ ID NO: 13 - DNA, 20 bp, Artificial Sequence
  mtDNA Primer sense 5'-3'
ccacttcatcttaccattta

SEQ ID NO: 14 - DNA, 20 bp, Artificial Sequence
  mtDNA Primer Antisense 5'-3'
atctgcatctgagtttaatc

SEQ ID NO: 15 - DNA, 23 bp, Artificial Sequence
  NRF1 Primer Sense 5'-3'
acagatagtcctgtctggggaaa

SEQ ID NO: 16 - DNA, 22 bp, Artificial Sequence
  NRF1 Primer Antisense 5'-3'
tggtacatgctcacagggatct

SEQ ID NO: 17 - DNA, 24 bp, Artificial Sequence
  PGC-1α Primer Sense 5'-3'
actatgaatcaagccactacagac

SEQ ID NO: 18 - DNA, 22 bp, Artificial Sequence
  PGC-1α Primer Antisense 5'-3'
ttcatccctcttgagcctttcg

SEQ ID NO: 19 - DNA, 20 bp, Artificial Sequence
  SESN2 Primer Sense 5'-3'
gcccctgagaagctccgcaa

SEQ ID NO: 20 - DNA, 20 bp, Artificial Sequence
  SESN2 Primer Antisense 5'-3'
gagttcggccagggaccagc

SEQ ID NO: 21 - DNA, 19 bp, Artificial Sequence
  SOD1 Primer Sense 5'-3'
ggcttctcgtcttgctctc

SEQ ID NO: 22 - DNA, 18 bp, Artificial Sequence
  SOD1 Primer Antisense 5'-3'
aactggttcaccgcttgc

SEQ ID NO: 23 - DNA, 20 bp, Artificial Sequence
  SOD2 Primer Sense 5'-3'
gcctcccagacctgccttac

SEQ ID NO: 24 - DNA, 22 bp, Artificial Sequence
  SOD2 Primer Antisense 5'-3'
gtggtacttctcctcggtggcg

SEQ ID NO: 25 - DNA, 23 bp, Artificial Sequence
  TBP Primer Sense 5'-3'
acccttcaccaatgactcctatg

SEQ ID NO: 26 - DNA, 21 bp, Artificial Sequence
  TBP Primer Antisense 5'-3'
tgactgcagcaaatcgcttgg

SEQ ID NO: 27 - DNA, 25 bp, Artificial Sequence
  Tfam Primer Sense 5'-3'
aagacctcgttcagcatataacatt

SEQ ID NO: 28 - DNA, 23 bp, Artificial Sequence
  Tfam Primer Antisense 5'-3'
ttttccaagcctcatttacaagc

SEQ ID NO: 29 - DNA, 25 bp, Artificial Sequence
  18S Primer Sense 5'-3'
ctgccctatcaactttcgatggtag

SEQ ID NO: 30 - DNA, 21 bp, Artificial Sequence
  18S Primer Antisense 5'-3'
ccgtttctcaggctccctctc